European Patent Specification EP 3 507 375 B1, published July 30, 2025. Title: GENETICALLY MODIFIED NON-HUMAN ANIMAL WITH  HUMAN OR CHIMERIC CTLA-4. Applicant: Beijing Biocytogen Co., Ltd. The sequence listing filed with the application follows.

SEQUENCE LISTING (71 sequences)

SEQ ID NO: 1 - DNA, 23 bp, Artificial Sequence
ggtcacctgtatggctgacatgg

SEQ ID NO: 2 - DNA, 23 bp, Artificial Sequence
tgaaggttgggtcacctgtatgg

SEQ ID NO: 3 - DNA, 23 bp, Artificial Sequence
acaggtgacccaaccttcagtgg

SEQ ID NO: 4 - DNA, 23 bp, Artificial Sequence
gacccaaccttcagtggtgttgg

SEQ ID NO: 5 - DNA, 23 bp, Artificial Sequence
agccaacaccactgaaggttggg

SEQ ID NO: 6 - DNA, 23 bp, Artificial Sequence
ctgctagccaacaccactgaagg

SEQ ID NO: 7 - DNA, 23 bp, Artificial Sequence
gtggtgttggctagcagccatgg

SEQ ID NO: 8 - DNA, 23 bp, Artificial Sequence
atggaaagctggcgacaccatgg

SEQ ID NO: 9 - DNA, 23 bp, Artificial Sequence
tgtgatggtgaatattcacatgg

SEQ ID NO: 10 - DNA, 23 bp, Artificial Sequence
accatcacacaacactgatgagg

SEQ ID NO: 11 - DNA, 23 bp, Artificial Sequence
acctcatcagtgttgtgtgatgg

SEQ ID NO: 12 - DNA, 23 bp, Artificial Sequence
acacaacactgatgaggtccggg

SEQ ID NO: 13 - DNA, 23 bp, Artificial Sequence
aggtccgggtgactgtgctgcgg

SEQ ID NO: 14 - DNA, 23 bp, Artificial Sequence
tctgccgcagcacagtcacccgg

SEQ ID NO: 15 - DNA, 23 bp, Artificial Sequence
tggcacagacctcagtcatttgg

SEQ ID NO: 16 - DNA, 23 bp, Artificial Sequence
actttgtgggcatgggcaacggg

SEQ ID NO: 17 - DNA, 23 bp, Artificial Sequence
ttgcccatgcccacaaagtatgg

SEQ ID NO: 18 - DNA, 23 bp, Artificial Sequence
ccgccatactttgtgggcatggg

SEQ ID NO: 19 - DNA, 23 bp, Artificial Sequence
atgcccacaaagtatggcggtgg

SEQ ID NO: 20 - DNA, 23 bp, Artificial Sequence
tacccaccgccatactttgtggg

SEQ ID NO: 21 - DNA, 23 bp, Artificial Sequence
ggactgagagctgttgacacggg

SEQ ID NO: 22 - DNA, 23 bp, Artificial Sequence
tgtcaacagctctcagtccttgg

SEQ ID NO: 23 - DNA, 23 bp, Artificial Sequence
gttcactctgctttcattaaagg

SEQ ID NO: 24 - DNA, 23 bp, Artificial Sequence
attaaaggtaccactgcagaagg

SEQ ID NO: 25 - DNA, 16 bp, Artificial Sequence
tgttggctagcagcca

SEQ ID NO: 26 - DNA, 20 bp, Artificial Sequence
taggtgttggctagcagcca

SEQ ID NO: 27 - DNA, 16 bp, Artificial Sequence
tggctgctagccaaca

SEQ ID NO: 28 - DNA, 20 bp, Artificial Sequence
aaactggctgctagccaaca

SEQ ID NO: 29 - DNA, 17 bp, Artificial Sequence
ccatactttgtgggcat

SEQ ID NO: 30 - DNA, 21 bp, Artificial Sequence
taggccatactttgtgggcat

SEQ ID NO: 31 - DNA, 17 bp, Artificial Sequence
atgcccacaaagtatgg

SEQ ID NO: 32 - DNA, 21 bp, Artificial Sequence
aaacatgcccacaaagtatgg

SEQ ID NO: 33 - DNA, 132 bp, Artificial Sequence
gaattctaatacgactcactatagggggtcttcgagaagacctgttttagagctagaaatagcaagttaaaataaggctagtccgttatcaacttgaaaaagtggcaccgagtcggtgcttttaaaggatcc

SEQ ID NO: 34 - DNA, 1933 bp, Mouse
ctacacatatgtagcacgtaccttggatcaaagctgtctatataaagtccccgagtctgtgtgggttcaaacacatctcaaggcttctggatcctgttgggttttactctgctccctgaggacctcagcacatttgccccccagccatggcttgtcttggactccggaggtacaaagctcaactgcagctgccttctaggacttggccttttgtagccctgctcactcttcttttcatcccagtcttctctgaagccatacaggtgacccaaccttcagtggtgttggctagcagccatggtgtcgccagctttccatgtgaatattcaccatcacacaacactgatgaggtccgggtgactgtgctgcggcagacaaatgaccaaatgactgaggtctgtgccacgacattcacagagaagaatacagtgggcttcctagattaccccttctgcagtggtacctttaatgaaagcagagtgaacctcaccatccaaggactgagagctgttgacacgggactgtacctctgcaaggtggaactcatgtacccaccgccatactttgtgggcatgggcaacgggacgcagatttatgtcattgatccagaaccatgcccggattctgacttcctcctttggatccttgtcgcagttagcttggggttgtttttttacagtttcctggtcactgctgtttctttgagcaagatgctaaagaaaagaagtcctcttacaacaggggtctatgtgaaaatgcccccaacagagccagaatgtgaaaagcaatttcagccttattttattcccatcaactgaaaggccgtttatgaagaagaaggagcatacttcagtctctaaaagctgaggcaatttcaactttccttttctctccagctatttttacctgtttgtatattttaaggagagtatgcctctctttaatagaaagctggatgcaaaattccaattaagcatactacaatttaaagctaaggagcatgaacagagagctgggatatttctgttgtgtcagaaccattttactaaaagcatcacttggaagcagcataaggatatagcattatggtgtggggtcaagggaacattagggaatggcacagcccaaagaaaggaagggggtgaaggaagagattatattgtacacatcttgtatttacctgagagatgtttatgacttaaataatttttaaatttttcatgctgttattttctttaacaatgtataattacacgaaggtttaaacatttattcacagagctatgtgacatagccagtggttccaaaggttgtagtgttccaagatgtatttttaagtaatattgtacatgggtgtttcatgtgctgttgtgtatttgctggtggtttgaatataaacactatgtatcagtgtcgtcccacagtgggtcctggggaggtttggctggggagcttaggacactaatccatcaggttggactcgaggtcctgcaccaactggcttggaaactagatgaggctgtcacagggctcagttgcataaaccgatggtgatggagtgtaaactgggtctttacactcattttattttttgtttctgcttttgttttcttcaatgatttgcaaggaaaccaaaagctggcagtgtttgtatgaacctgacagaacactgtcttcaaggaaatgcctcattcctgagaccagtaggtttgtttttttaggaagttccaatactaggaccccctacaagtactatggctcctcgaaaacacaaagttaatgccacaggaagcagcagatggtaggatgggatgcacaagagttcctgaaaactaacactgttagtgttttttttttaactcaatattttccatgaaaatgcaaccacatgtataatatttttaattaaataaaagtttcttgtgattgtttt

SEQ ID NO: 35 - protein, 223 aa, Mouse
MACLGLRRYKAQLQLPSRTWPFVALLTLLFIPVFSEAIQVTQPSVVLASSHGVASFPCEYSPSHNTDEVRVTVLRQTNDQMTEVCATTFTEKNTVGFLDYPFCSGTFNESRVNLTIQGLRAVDTGLYLCKVELMYPPPYFVGMGNGTQIYVIDPEPCPDSDFLLWILVAVSLGLFFYSFLVTAVSLSKMLKKRSPLTTGVYVKMPPTEPECEKQFQPYFIPIN

SEQ ID NO: 36 - DNA, 2033 bp, Human
cttctgtgtgtgcacatgtgtaatacatatctgggatcaaagctatctatataaagtccttgattctgtgtgggttcaaacacatttcaaagcttcaggatcctgaaaggttttgctctacttcctgaagacctgaacaccgctcccataaagccatggcttgccttggatttcagcggcacaaggctcagctgaacctggctaccaggacctggccctgcactctcctgttttttcttctcttcatccctgtcttctgcaaagcaatgcacgtggcccagcctgctgtggtactggccagcagccgaggcatcgccagctttgtgtgtgagtatgcatctccaggcaaagccactgaggtccgggtgacagtgcttcggcaggctgacagccaggtgactgaagtctgtgcggcaacctacatgatggggaatgagttgaccttcctagatgattccatctgcacgggcacctccagtggaaatcaagtgaacctcactatccaaggactgagggccatggacacgggactctacatctgcaaggtggagctcatgtacccaccgccatactacctgggcataggcaacggaacccagatttatgtaattgatccagaaccgtgcccagattctgacttcctcctctggatccttgcagcagttagttcggggttgtttttttatagctttctcctcacagctgtttctttgagcaaaatgctaaagaaaagaagccctcttacaacaggggtctatgtgaaaatgcccccaacagagccagaatgtgaaaagcaatttcagccttattttattcccatcaattgagaaaccattatgaagaagagagtccatatttcaatttccaagagctgaggcaattctaacttttttgctatccagctatttttatttgtttgtgcatttggggggaattcatctctctttaatataaagttggatgcggaacccaaattacgtgtactacaatttaaagcaaaggagtagaaagacagagctgggatgtttctgtcacatcagctccactttcagtgaaagcatcacttgggattaatatggggatgcagcattatgatgtgggtcaaggaattaagttagggaatggcacagcccaaagaaggaaaaggcagggagcgagggagaagactatattgtacacaccttatatttacgtatgagacgtttatagccgaaatgatcttttcaagttaaattttatgccttttatttcttaaacaaatgtatgattacatcaaggcttcaaaaatactcacatggctatgttttagccagtgatgctaaaggttgtattgcatatatacatatatatatatatatatatatatatatatatatatatatatatatatatatatattttaatttgatagtattgtgcatagagccacgtatgtttttgtgtatttgttaatggtttgaatataaacactatatggcagtgtctttccaccttgggtcccagggaagttttgtggaggagctcaggacactaatacaccaggtagaacacaaggtcatttgctaactagcttggaaactggatgaggtcatagcagtgcttgattgcgtggaattgtgctgagttggtgttgacatgtgctttggggcttttacaccagttcctttcaatggtttgcaaggaagccacagctggtggtatctgagttgacttgacagaacactgtcttgaagacaatggcttactccaggagacccacaggtatgaccttctaggaagctccagttcgatgggcccaattcttacaaacatgtggttaatgccatggacagaagaaggcagcaggtggcagaatggggtgcatgaaggtttctgaaaattaacactgcttgtgtttttaactcaatattttccatgaaaatgcaacaacatgtataatatttttaattaaataaaaatctgtggtggtcgttttaaaaaaaaaaaaaaaaaaaaaaaaaaaaaaaaaaaaaaaaaaaaaaaaaaaaaaaaaa

SEQ ID NO: 37 - protein, 223 aa, Human
MACLGFQRHKAQLNLATRTWPCTLLFFLLFIPVFCKAMHVAQPAVVLASSRGIASFVCEYASPGKATEVRVTVLRQADSQVTEVCAATYMMGNELTFLDDSICTGTSSGNQVNLTIQGLRAMDTGLYICKVELMYPPPYYLGIGNGTQIYVIDPEPCPDSDFLLWILAAVSSGLFFYSFLLTAVSLSKMLKKRSPLTTGVYVKMPPTEPECEKQFQPYFIPIN

SEQ ID NO: 38 - DNA, 361 bp, Artificial Sequence
ccatgtcagccatacaggtggcccagcctgctgtggtactggccagcagccgaggcatcgccagctttgtgtgtgagtatgcatctccaggcaaagccactgaggtccgggtgacagtgcttcggcaggctgacagccaggtgactgaagtctgtgcggcaacctacatgatggggaatgagttgaccttcctagatgattccatctgcacgggcacctccagtggaaatcaagtgaacctcactatccaaggactgagggccatggacacgggactctacatctgcaaggtggagctcatgtacccaccgccatactacctgggcataggcaacgggacgcagatttatgtcattggtga

SEQ ID NO: 39 - DNA, 672 bp, Artificial Sequence
atggcttgtcttggactccggaggtacaaagctcaactgcagctgccttctaggacttggccttttgtagccctgctcactcttcttttcatcccagtcttctctgaagccatacaggtggcccagcctgctgtggtactggccagcagccgaggcatcgccagctttgtgtgtgagtatgcatctccaggcaaagccactgaggtccgggtgacagtgcttcggcaggctgacagccaggtgactgaagtctgtgcggcaacctacatgatggggaatgagttgaccttcctagatgattccatctgcacgggcacctccagtggaaatcaagtgaacctcactatccaaggactgagggccatggacacgggactctacatctgcaaggtggagctcatgtacccaccgccatactacctgggcataggcaacgggacgcagatttatgtcattgatccagaaccatgcccggattctgacttcctcctttggatccttgtcgcagttagcttggggttgtttttttacagtttcctggtcactgctgtttctttgagcaagatgctaaagaaaagaagtcctcttacaacaggggtctatgtgaaaatgcccccaacagagccagaatgtgaaaagcaatttcagccttattttattcccatcaactga

SEQ ID NO: 40 - DNA, 1933 bp, Artificial Sequence
ctacacatatgtagcacgtaccttggatcaaagctgtctatataaagtccccgagtctgtgtgggttcaaacacatctcaaggcttctggatcctgttgggttttactctgctccctgaggacctcagcacatttgccccccagccatggcttgtcttggactccggaggtacaaagctcaactgcagctgccttctaggacttggccttttgtagccctgctcactcttcttttcatcccagtcttctctgaagccatacaggtggcccagcctgctgtggtactggccagcagccgaggcatcgccagctttgtgtgtgagtatgcatctccaggcaaagccactgaggtccgggtgacagtgcttcggcaggctgacagccaggtgactgaagtctgtgcggcaacctacatgatggggaatgagttgaccttcctagatgattccatctgcacgggcacctccagtggaaatcaagtgaacctcactatccaaggactgagggccatggacacgggactctacatctgcaaggtggagctcatgtacccaccgccatactacctgggcataggcaacgggacgcagatttatgtcattgatccagaaccatgcccggattctgacttcctcctttggatccttgtcgcagttagcttggggttgtttttttacagtttcctggtcactgctgtttctttgagcaagatgctaaagaaaagaagtcctcttacaacaggggtctatgtgaaaatgcccccaacagagccagaatgtgaaaagcaatttcagccttattttattcccatcaactgaaaggccgtttatgaagaagaaggagcatacttcagtctctaaaagctgaggcaatttcaactttccttttctctccagctatttttacctgtttgtatattttaaggagagtatgcctctctttaatagaaagctggatgcaaaattccaattaagcatactacaatttaaagctaaggagcatgaacagagagctgggatatttctgttgtgtcagaaccattttactaaaagcatcacttggaagcagcataaggatatagcattatggtgtggggtcaagggaacattagggaatggcacagcccaaagaaaggaagggggtgaaggaagagattatattgtacacatcttgtatttacctgagagatgtttatgacttaaataatttttaaatttttcatgctgttattttctttaacaatgtataattacacgaaggtttaaacatttattcacagagctatgtgacatagccagtggttccaaaggttgtagtgttccaagatgtatttttaagtaatattgtacatgggtgtttcatgtgctgttgtgtatttgctggtggtttgaatataaacactatgtatcagtgtcgtcccacagtgggtcctggggaggtttggctggggagcttaggacactaatccatcaggttggactcgaggtcctgcaccaactggcttggaaactagatgaggctgtcacagggctcagttgcataaaccgatggtgatggagtgtaaactgggtctttacactcattttattttttgtttctgcttttgttttcttcaatgatttgcaaggaaaccaaaagctggcagtgtttgtatgaacctgacagaacactgtcttcaaggaaatgcctcattcctgagaccagtaggtttgtttttttaggaagttccaatactaggaccccctacaagtactatggctcctcgaaaacacaaagttaatgccacaggaagcagcagatggtaggatgggatgcacaagagttcctgaaaactaacactgttagtgttttttttttaactcaatattttccatgaaaatgcaaccacatgtataatatttttaattaaataaaagtttcttgtgattgtttt

SEQ ID NO: 41 - protein, 223 aa, Artificial Sequence
MACLGLRRYKAQLQLPSRTWPFVALLTLLFIPVFSEAIQVAQPAVVLASSRGIASFVCEYASPGKATEVRVTVLRQADSQVTEVCAATYMMGNELTFLDDSICTGTSSGNQVNLTIQGLRAMDTGLYICKVELMYPPPYYLGIGNGTQIYVIDPEPCPDSDFLLWILVAVSLGLFFYSFLVTAVSLSKMLKKRSPLTTGVYVKMPPTEPECEKQFQPYFIPIN

SEQ ID NO: 42 - DNA, 1518 bp, Artificial Sequence
atgagcaaagggtgcttgcagaaagtctctgatagtagagatgaaggctaggcagacacctgctgtttcacccgctaagctgatggagtaaccatggcaactgccaccatattgttctcttttctgaggacagatgctaatcagtacaggtgctttcagaagagactagggtatctatatagcctggtttatggataggagaggtggtcttggaaactaagcctggggtagtattcaagattgcaatacactgaaaactaattattgtcttgtttttacaatctatgttagtaaactaccaatgacattgttcagtttaagttttgggtgtaatcttcaatactgaccggaaaacatccaggttagttatgaaaaggcaatatgacagaaagccacttttgtgtgctgagagtacaacccgagatcgtgtgtattctaggcaagcactctaccaccgacctacatctccagcccttctgcctgtggttctttgtcttgtaaagcaatgtcttgttgtttagctgatgctggccttgcacttgctatgtagccttcatctgctggctgctaggactgcagatttgtaccaccaataccggactgcaaacccactaatttctaatgatgaaggcatgtttgtatagagagctggactcctttcttctgtagtatacagggaggaaagagaaaacaacaaaaacagcagcagcagcagcagcaacaacaacaacaacaaaaaccccaaggacaaggaaagtgttaagtgaaggaaagaagggaggcagaagaggtggcagggaagcaggggaagcccacagaagttaaagcagggttgtctcaacccagagaggaaatgaccctggtgccctcagctctgtggcttccttgactgatgtatacaccactctaccacagtgatgccaggaaaagggtgaccaatgcattgacctgaggttcaactgctcctggttgacagaggtacgcttataaataagtaggtaggaaaattttgaagcttactttgagagatgaggcaaggttctgcacctcaagctccaggaatgtctcgactgccattcactatgtttcctgcgtgatatagttctattatcaccaaagaaggcgctgtactgacatgtaggctacccccttttcttactgcaggggagaataaatgaaaggaagaattatttgccaaaatgacacattttatgagagccagatcttctttttgctataccagtattctccttgccatagccaactgtcttcaataaactatcaataaggggatcttggagagtgactgactacagctgaaagatgggaagtggagtgccagggtggatgggtggagaggcaaagggtgaagggagtgatgagtttgttgaggggtgagcttgcaggagttcatccaagatgaacctcccctggcctcaggtgtggcctaatagttcaaaccgtggatgatcatgagcccactaagtgccctttggactttccatgtcagccatacag

SEQ ID NO: 43 - DNA, 54 bp, Artificial Sequence
tttaagaaggagatatacatgctcgagatgagcaaagggtgcttgcagaaagtc

SEQ ID NO: 44 - DNA, 45 bp, Artificial Sequence
accacagcaggctgggccacctgtatggctgacatggaaagtcca

SEQ ID NO: 45 - DNA, 312 bp, Human
gtggcccagcctgctgtggtactggccagcagccgaggcatcgccagctttgtgtgtgagtatgcatctccaggcaaagccactgaggtccgggtgacagtgcttcggcaggctgacagccaggtgactgaagtctgtgcggcaacctacatgatggggaatgagttgaccttcctagatgattccatctgcacgggcacctccagtggaaatcaagtgaacctcactatccaaggactgagggccatggacacgggactctacatctgcaaggtggagctcatgtacccaccgccatactacctgggcata

SEQ ID NO: 46 - DNA, 44 bp, Artificial Sequence
tggactttccatgtcagccatacaggtggcccagcctgctgtgg

SEQ ID NO: 47 - DNA, 41 bp, Artificial Sequence
taaatctgcgtcccgttgcctatgcccaggtagtatggcgg

SEQ ID NO: 48 - DNA, 973 bp, Artificial Sequence
ggcaacgggacgcagatttatgtcattggtgagcaaagccattccactaagaacaagtctgttgcattattattgtctttacaccagaatagttttgttccttggtttggagtccttcatagttaggtctgtgatgcatagctaggaattccctagtagatagtagtcttgcttatactgagaagttacataaccatcactctgattgcaatgaaacgcatttggggatgtgttttttatactgcttgctgatagtctaggacacttgttcttgaagtttagtcttgtccctttgatggcactctgggaaagtcatgtattaaataagtagccagacttccctatagtttaccaatacaagttagggttgactagcaaaacctggaacctctaacttccttttactacccatgaggaactaggaccccacaattggaaactctctcaggaggttgatgcttcgtcttctgttgcagatccagaaccatgcccggattctgacttcctcctttggatccttgtcgcagttagcttggggttgtttttttacagtttcctggtcactgctgtttctttgagcaagatggtgagtgtgatgttgacgtttccccacagttaatggggatacttttagttgtaccctactgaccaattggtgttgagttgaagcaataaacaaggagcaggaaggatagggtaaagaacacgctagaaccccatgcacttgccttagaggtttcgggatgactaatactgtacgtgagcatgtttgacagtgaatgtttgtgtgcttctgagcagggtttcagtttgagtaactgtttgaacaacatggagcagctgttttggttgtcactgtcatggcaatgtccttaatcctaggacacacagcagtctctgggcaaccctttctagttagaaccacctagatggatttttgtcctttaccaagcaccatctcttggtccctctt

SEQ ID NO: 49 - DNA, 42 bp, Artificial Sequence
cgccatactacctgggcataggcaacgggacgcagatttatg

SEQ ID NO: 50 - DNA, 52 bp, Artificial Sequence
ttgttagcagccggatctcaggcggccgcaagagggaccaagagatggtgct

SEQ ID NO: 51 - DNA, 29 bp, Artificial Sequence
gaaaggctaataccaggcttgttatgtgc

SEQ ID NO: 52 - DNA, 28 bp, Artificial Sequence
tcaactcattccccatcatgtaggttgc

SEQ ID NO: 53 - DNA, 25 bp, Artificial Sequence
gagtatgcatctccaggcaaagcca

SEQ ID NO: 54 - DNA, 25 bp, Artificial Sequence
cactgagctagggagggcatcaagg

SEQ ID NO: 55 - DNA, 25 bp, Artificial Sequence
tgtgttaaagcaacacagcgtggtc

SEQ ID NO: 56 - DNA, 25 bp, Artificial Sequence
aactgttgttgccgtttggtccttg

SEQ ID NO: 57 - DNA, 25 bp, Artificial Sequence
agaagaccattgcttttggctgttt

SEQ ID NO: 58 - DNA, 25 bp, Artificial Sequence
acatggaaaagtgcagaactaaaga

SEQ ID NO: 59 - DNA, 19 bp, Artificial Sequence
accccttgaggttagccct

SEQ ID NO: 60 - DNA, 23 bp, Artificial Sequence
ttgtagaacagctatacgaccca

SEQ ID NO: 61 - DNA, 21 bp, Artificial Sequence
atactgtgctaacaggcctca

SEQ ID NO: 62 - DNA, 23 bp, Artificial Sequence
acccattgtcattaggaagcact

SEQ ID NO: 63 - DNA, 45 bp, Artificial Sequence
gcatcaagcttggtaccgatacagctgaaagatgggaagtggagt

SEQ ID NO: 64 - DNA, 45 bp, Artificial Sequence
acttaatcgtggaggatgatcacatccccaaatgcgtttcattgc

SEQ ID NO: 65 - DNA, 25 bp, Artificial Sequence
ccatcacacaacactgatgaggtcc

SEQ ID NO: 66 - DNA, 25 bp, Artificial Sequence
cacatccccaaatgcgtttcattgc

SEQ ID NO: 67 - DNA, 25 bp, Artificial Sequence
acagctgaaagatgggaagtggagt

SEQ ID NO: 68 - DNA, 25 bp, Artificial Sequence
cttccacatgagcgtggtcagggcc

SEQ ID NO: 69 - DNA, 25 bp, Artificial Sequence
ccaagggactattttagatgggcag

SEQ ID NO: 70 - DNA, 26 bp, Artificial Sequence
gaagctacaagctcctaggtaggggg

SEQ ID NO: 71 - DNA, 23 bp, Artificial Sequence
acgggttggctcaaaccattaca